European Patent Application EP 4 155 394 A1, published March 29, 2023. Title: USE OF LYTIC POLYSACCHARIDE MONOOXYGENASES, ENZYMATIC COMPOSITION CONTAINING SAME, AND DEGRADATION METHOD FOR PLASTIC POLYMERS. Applicant: CNPEM - CENTRO NACIONAL DE PESQUISA EM ENERGIA E MATERIAIS. Application EP. The sequence listing filed with the application follows.

SEQUENCE LISTING (5 sequences)

SEQ ID NO: 1 - DNA, 672 bp, Kitasatospora papulosa
  source 1..672: mol_type = genomic DNA
atgaggaaaaattgtcatgagcgcgtcagtttagtcggttgggcgcggcgcgtcggtggcgtgtgcgtcgccgccgtcctctgtctgctcccctggacgggcaccgcgagcgcccacggttccgtcgtcgaccccgcttcccgcaactacggctgctggctgcgctggggcgacgacttccagaacccggccatggagcaggaggaccccatgtgctggcaggcctggcaggccgacccgaacgccatgtggaactggaacggcctgtaccgcaacggctcgggcggcgacttccccgcggccgtgcccgacgggcaactgtgcagcggtggccgcacggagagcggacggtacgactcgctcgactccgtcggtgcgtggaagaccacggacatcaccgatgacttcaccgtgaagctgtacgaccaggccagtcacggcgcggactacttccaggtgtacgtcacccggcagggattcgatcctgccgcggaggcgctgacctggagcgacctccaactggtcgccgagaccggccgctacgcgccgagccagaactacgagatccccgtgaccacctcggggctcagcggccggcacgtggtctacacgatctggcaggcgtcgcacatggaccagacgtacttcctgtgcagtgacgtgaacttcacc

SEQ ID NO: 2 - protein, 224 aa, Kitasatospora papulosa
MRKNCHERVSLVGWARRVGGVCVAAVLCLLPWTGTASAHGSVVDPASRNYGCWLRWGDDFQNPAMEQEDPMCWQAWQADPNAMWNWNGLYRNGSGGDFPAAVPDGQLCSGGRTESGRYDSLDSVGAWKTTDITDDFTVKLYDQASHGADYFQVYVTRQGFDPAAEALTWSDLQLVAETGRYAPSQNYEIPVTTSGLSGRHVVYTIWQASHMDQTYFLCSDVNFT

SEQ ID NO: 3 - DNA, 741 bp, Aspergillus fischeri
  source 1..741: mol_type = genomic DNA
atgtctgtctctaagattgcagctgttcttctcagctcggccgctctggttgctggtcacggattcgtgtcgggtgccgttgttgatggcaaatactacactggatacctcgtcaaccaatacccttacatgagcagccctcctgagagcatcggttggtctgaaaccgctaccgatctgggtttcgtcgacggtagcggctactctagcggcgacatcatctgccacaagagtgctaagaatggtgccatctctgccgagatcaaggccggtggaaaggttgaattccaatggactgaatggcctgaatctcaccacggaccggtcattacctacatggccaactgcaatggtgattgcgcctcagttgacaagaccagtctggaattcttcaagattgatgagagtggtctgatcagtgactctaatgttcctggcacctgggcctccgacaacctaatcgccaacaacaacagctggacggtgactgttcccagctccatcgccgctggtaactatgtcatgcgtcacgaaatcattgccctccactccgctggaaaccagaacggtgcccagaactaccctcagtgcatcaaccttaaggtcaccggtggtggcagcgacaagcctgcaggtaccctcggcactgcgctctacaagaacactgacgccggcatccttgtcaatatctaccagagcctgagctcctatgacattcctggtcccgctctctactctggc

SEQ ID NO: 4 - DNA, 750 bp, Aspergillus fischeri
  source 1..750: mol_type = genomic DNA
atgaaatacctgctgccgaccgctgctgctggtctgctgctcctcgctgcccagccggcgatggcccacggtttcgtttctggtgcggttgttgacggtaaatactacaccggttacctggttaaccagtacccgtacatgtcttctccgccggaatctatcggttggtctgaaaccgcgaccgacctgggtttcgttgacggttctggttactcttctggtgacatcatctgccacaaatctgcgaaaaacggtgcgatctctgcggaaatcaaagcgggtggtaaagttgaattccagtggaccgaatggccggaatctcaccacggtccggttatcacctacatggcgaactgcaacggtgactgcgcgtctgttgacaaaacctctctggaattcttcaaaatcgacgaatctggtctgatctctgactctaacgttccgggtacctgggcgtctgacaacctgatcgcgaacaacaactcttggaccgttaccgttccgtcttctatcgcggcgggtaactacgttatgcgtcacgaaatcatcgcgctgcactctgcgggtaaccagaacggtgcgcagaactacccgcagtgcatcaacctgaaagttaccggtggtggttctgacaaaccggcgggtaccctgggtaccgcgctgtacaaaaacaccgacgcgggtatcctggttaacatctaccagtctctgtcttcttacgacatcccgggtccggcgctgtactctggt

SEQ ID NO: 5 - protein, 247 aa, Aspergillus fischeri
MSVSKIAAVLLSSAALVAGHGFVSGAVVDGKYYTGYLVNQYPYMSSPPESIGWSETATDLGFVDGSGYSSGDIICHKSAKNGAISAEIKAGGKVEFQWTEWPESHHGPVITYMANCNGDCASVDKTSLEFFKIDESGLISDSNVPGTWASDNLIANNNSWTVTVPSSIAAGNYVMRHEIIALHSAGNQNGAQNYPQCINLKVTGGGSDKPAGTLGTALYKNTDAGILVNIYQSLSSYDIPGPALYSG